European Patent Specification EP 4 392 563 B1, published February 26, 2025. Title: A Novel Type of CRISPR/Cas System. Applicant: SNIPR Biome ApS. The sequence listing filed with the application follows.

SEQUENCE LISTING (70 sequences)

SEQ ID NO: 1 - protein, 263 aa, synthetic construct
LNHPVESVYSALTSILLPYMGEPVPVQRNCSCCGRAPSEFDGVGFELVNAYRERVVHCRPCQTFFVSAPELMGVENPKKPTTGQKFGMWSGVGAVINVEDNSSVLLAPQGVVNKLPEHFFDHVEVITATSGQHLEYLFNTELKFPLIYIQNFGVKTYELVRSLRVSLSADAIYTCADQLLTRQNEVLYMLDLTKAKELHQEIKNYSKKEIDIFIRTVTLLAYSRITPEAASNEFKKNNLIPLLLLLPTDPHQRLSILHLLKKV

SEQ ID NO: 2 - protein, 188 aa, synthetic construct
MIYYDNAFRLRIRHTSVYQIHQHLDFFMQERKGEKLPYSFKIFPGTGDDSLLLVRTATALELPGEKKRELILSEGHEIKFITSMAIFHKGTKSEGRGRRQFAPSEEASYQLALTKLAKAGFKPGQIVVSGPKFVHIVKGNAGRGFTLPVFTVQGTAIISNQQEAEVGIVYGVGPKRVFGCGFMHLAGQ

SEQ ID NO: 3 - protein, 624 aa, synthetic construct
MNTSAVFESAGLSLRKVQQDYIEAAAGALTQDHKVALISAETGVGKTLGYLVPALLILLKNPEAKFVIATNSHALMHQIFRSDRPLLEQIAEQCGIKVTFSRLMGKANYVSLEKVRGLLLMDEFTDLDTVKVLEKLANWSKPLVEFEEEYGELPAQITPEMVTYSIWDDIQDIDDIRLNALSANFIVTTHAMVMVDCMCNHRILGDKENMYLIIDEADIFVDMLEVWKQRRFNLRELTSAFNEHIPRNGVHVIDQLMNDVTSIAGDLHFCSTPAAVALFDNSFNALSKVGREIKNEAARKAFFDCIYSWEMLGLSGGQKGVGVSNKRREPALIAVNPFIGMNVGRYCTQWRSALLTSATLSITSTPETGMEWLCKALGLTSDTISIRKIFSPDVYGSMKLTIAGADFPKVFNDPKEQIFSGQWLKAVVEQLSCIQGPALVLTASHYETRMIANQLGEVSQPVYIQKAGQALSEIIKQYQEIPGILISAGASVGVSPRGENGEQIFQDLIITRIPFLPPDRMKAESLYGYLKERGYSRTFEAVNRNIYLDNLRKVIRKAKQSIGRGIRSENDTVRIIILDPRFPEPTDLSSKHRSLEHIIPVRFRRAYRSCEILSPAYCEEDIQC

SEQ ID NO: 4 - protein, 235 aa, synthetic construct
VLNFKPYRVIMSSLTPVVISGIAPSLDGILYEALSQAIPSNEPGVVLARLKEILLFNDELGVFHASSLRFGITPEQGIGATTSVRCDYLSPEKLSTAMFSPRIHRGVFTRVLLTGGPTKRRMTTRPAYSAPYLTFDFVGSSEAVEILLNHAHVGVGYDFFSAANGEFNNVTILPLDIDTSISNEGMALRPVPVNSGLNGIKGVSPLIPPYFVGEKLNIVHPAPVRTQLISSLLRG

SEQ ID NO: 5 - protein, 343 aa, synthetic construct
MRTLNFNGKISTLEPLTVTVKNAVSTSGHRLPRNGGFNAAPYFPGTSIRGTLRHAAHKVIVDRVGLNADGKSSFDLAEHFMLAQGVDINGEAETFAPGEINAGAELRSKNPLISLFGRWGLSGKVGIGNAIPDGDNQWGMFGGGARSIMFQRDESLMEFLETDQVDRLERLLEEQAEASVDISQIKTEQDALKKAMKSADKDTKAELQIKVRELDEKIQARKDQKQESRESIRRPIDPYEAFITGAELSHRMSIKNATDEEAGLFISALIRFAAEPRFGGHANHNCGLVEAHWTVTTWKPGELVPVTLGEIVITPNGVEITGDELFAMVKAFNENQSFDFTAR

SEQ ID NO: 6 - DNA, 29 bp, synthetic construct
  source 1..29: mol_type = other DNA
gtattccccccgtgtgcgggggttatcgg

SEQ ID NO: 7 - DNA, 748 bp, synthetic construct
  source 1..748: mol_type = other DNA
ttgaatcatcctgtagagtcagtatatagcgctctgacgagtattttattgccctatatgggtgagcctgtgcctgtgcaacgaaattgctcatgctgcggcagagcgccctcagagttcgacggggtaggcttcgagctggtcaacgcctacagggaacgtgttgtgcattgccgtccttgccagacattttttgtttctgctccagaactgatgggcgtggagaaccccaaaaaaccaacaaccggccagaaatttggcatgtggtctggtgttggggctgttattaacgttgaagacaattcttcggttcttttagcccctcagggagtggtcaataaactacctgagcattttttcgatcacgtagaagtcatcacggccaccagcggtcagcacctggaatacctgtttaacaccgaacttaaattcccgctgatttatattcaaaacttcggcgtgaaaacctacgagcttgttcgctcactgcgggtcagtctgagtgccgacgcaatttatacctgtgccgatcaactactgacccggcagaacgaagtcctttacatgctggatttaacaaaggctaaagaactccatcaggaaataaaaaactactccaaaaaagagatagacatctttatcagaacagtaaccctgctggcctattcgcggataactcctgaagctgcctcgaatgagtttaagaaaaacaacctcattccgttactgctgcttctgccgactgatc

SEQ ID NO: 8 - DNA, 567 bp, synthetic construct
  source 1..567: mol_type = other DNA
atgatttactacgataatgcgtttcggttgcgtatccgtcacacaagtgtttaccagatccaccagcacctggattttttcatgcaggaacgtaagggagagaagctgccgtactcttttaaaatttttcccggtaccggggatgattcgttactcctggtccgcacagccacagctctggagttgccaggggagaaaaaaagagagcttattctctctgagggccatgaaatcaagttcattacgtcaatggccatctttcataaaggaacaaagtcagaaggccgtggccgacgccagtttgctccatccgaagaggctagttatcagttggccctcaccaaattagcgaaggctggttttaaacccggtcaaatcgtcgtcagtggcccgaaattcgtccatatcgtcaaaggaaatgctggacgcggttttacgctacccgtattcacggtacagggtaccgccataatcagcaatcaacaggaagctgaagttggaatcgtttatggcgtaggccctaaacgcgtatttggttgcggtttcatgcatctggcggggcagtag

SEQ ID NO: 9 - DNA, 1871 bp, synthetic construct
  source 1..1871: mol_type = other DNA
atgaatacatcagcggtatttgagtctgccggattgtcgttacgtaaggtccaacaggattatatcgaggctgcagctggtgcgctgactcaggatcataaagttgcactgattagtgctgaaacaggtgtaggaaaaacgctgggctatctggtaccggcgcttctgattctgctgaaaaacccagaggcaaaatttgtgatagccacgaattctcatgccctgatgcaccagatattcagaagcgatcgtcctctccttgaacagatagctgaacaatgcggcataaaagttactttttcccggcttatggggaaagcaaattacgtatccctggagaaagtacgtggactgttactcatggacgaatttaccgatctggatacggttaaggtccttgaaaaactcgctaactggtcaaaacctctggttgagtttgaagaagagtatggtgaactgccagcgcagatcacgccagagatggtcacctactccatctgggatgatatacaggacattgatgatattcgcctgaatgctctcagtgctaactttatagttacgacccatgcgatggtaatggtcgactgtatgtgtaatcaccgcatcctcggtgacaaagaaaatatgtacctcattattgatgaggcagacatttttgtagatatgcttgaggtctggaaacagcggcgcttcaacctcagagagttgaccagtgcgttcaatgaacatattccacgtaatggcgtgcatgtcatcgaccagttaatgaacgacgtgacttcgatagcgggcgatctgcatttttgtagtacgcctgcagcggttgccttgtttgacaatagctttaacgccttatcaaaggtagggcgggaaataaaaaatgaagcggcccggaaagctttctttgactgtatctacagctgggaaatgctcggattgtccggggggcaaaagggtgtaggcgtttccaataaacgtcgtgaaccagccctgatcgctgtaaacccgtttatcgggatgaatgtgggcagatactgcactcaatggcgtagtgcgttactgacgtcggctacgctctcaattaccagtaccccagagaccggaatggagtggttatgtaaagctctggggttaaccagcgatacgatttcaatcaggaaaatattctccccagacgtctatggctcaatgaagctgaccatcgccggtgctgattttccaaaggtgttcaatgacccgaaagaacagatattttcaggtcaatggttaaaggcagtagttgaacaattgtcctgtattcaggggccagctctggtattaactgccagccattatgaaaccaggatgattgccaatcagctgggtgaggtctcgcaaccagtttatattcagaaagcaggtcaggccctgtccgaaattattaaacagtatcaggagataccagggattcttatttctgccggtgcttctgttggtgtgagcccacgaggcgagaatggggaacagattttccaggatttaatcattacccggatacctttcttacctccggacagaatgaaggctgaaagcctttatgggtatctgaaggaacgaggctatagtcgtacctttgaggcagttaaccgtaacatctacctggataatttgcggaaagttattcgtaaagcaaagcagtctatagggcgggggattcgtagtgaaaatgataccgtcaggataattatcctcgatccgcgtttcccggaacctactgacctttcgtctaaacatcggtcgcttgaacacattattcccgttcgatttcgtcgtgcatatcgttcgtgtgaaattttatctccggcgtattgtgaagaggatatccagtg

SEQ ID NO: 10 - DNA, 708 bp, synthetic construct
  source 1..708: mol_type = other DNA
gtgttaaattttaaaccgtatcgggtcatcatgtcttctctgacaccggtggtcatcagtgggatagccccatcgctggacggcattctgtatgaagcactgtctcaggcgatacccagtaacgagccaggagtcgtattggctcgtcttaaggaaatacttctattcaacgatgaactgggtgttttccatgcttcatctctacgttttggcataacgcccgaacaggggattggggcgacaacaagcgtacgttgcgattatctcagtcccgaaaaactgagcactgcaatgttctctcctcgtatccacaggggggtgtttacgcgtgtcctcctgaccgggggccccacgaagagaaggatgacaacccgtccagcttattctgcaccctatttaacgtttgattttgtcggctcttctgaggctgtagaaatactgcttaaccatgcccatgttggcgttggttatgactttttctctgcagctaatggagagtttaacaatgtgacaattcttcctctcgatatcgacacgagtatatccaacgagggtatggcattgcgtccggtacctgttaattcgggtctgaatggtatcaaaggagtatcaccacttattcctccctatttcgttggtgaaaagctaaacattgtccacccagcaccagttcgtactcaattgatttcttctttattgcgaggctaa

SEQ ID NO: 11 - DNA, 1032 bp, synthetic construct
  source 1..1032: mol_type = other DNA
atgagaactttaaacttcaacggtaaaatttcgactctggaaccactgactgtaacagtaaaaaatgcggtctcaacttccggccatcgcttgcctcgtaacggtggattcaatgcagccccgtactttccaggtaccagcattcggggaactcttcgtcatgctgcgcataaggtcattgtcgatcgtgtgggccttaatgcagacggaaaatcatccttcgacctggcagaacatttcatgctggcccagggggtggatatcaatggtgaagccgaaaccttcgcgccaggtgaaatcaatgctggtgctgaactacgtagcaaaaacccgttaatcagcttgtttggtcgttggggattaagcggcaaagttggtatagggaatgctatcccggatggtgataaccagtgggggatgtttggtggtggtgcccgctcaattatgtttcagcgtgacgaaagtctgatggagtttcttgagacagaccaggttgatcgtcttgaacgcctgctcgaggaacaggctgaggcaagtgtggatatctctcagatcaaaacagagcaagatgcactcaaaaaggcgatgaagtcggctgataaagacaccaaagctgagcttcaaatcaaagtacgggagctcgatgaaaaaattcaggcccgcaaagatcagaagcaggaatctcgcgagtcaattcgccgcccgattgacccgtatgaagcgtttatcaccggcgcagaactcagccatcgcatgagtattaaaaatgcgactgatgaggaagcagggcttttcatttctgcattaatccgctttgcagccgaaccacgttttggcggtcatgcgaatcataactgcggtctggtggaggctcactggacagttacgacctggaagccgggtgaactggtaccagttacacttggagaaatcgtcatcacaccgaatggtgttgagattaccggggacgagttgtttgctatggtaaaggcattcaatgaaaatcaatcttttgatttcactgcccgctaa

SEQ ID NO: 12 - DNA, 5636 bp, synthetic construct
  source 1..5636: mol_type = other DNA
ttgaatcatcctgtagagtcagtatatagcgctctgacgagtattttattgccctatatgggtgagcctgtgcctgtgcaacgaaattgctcatgctgcggcagagcgccctcagagttcgacggggtaggcttcgagctggtcaacgcctacagggaacgtgttgtgcattgccgtccttgccagacattttttgtttctgctccagaactgatgggcgtggagaaccccaaaaaaccaacaaccggccagaaatttggcatgtggtctggtgttggggctgttattaacgttgaagacaattcttcggttcttttagcccctcagggagtggtcaataaactacctgagcattttttcgatcacgtagaagtcatcacggccaccagcggtcagcacctggaatacctgtttaacaccgaacttaaattcccgctgatttatattcaaaacttcggcgtgaaaacctacgagcttgttcgctcactgcgggtcagtctgagtgccgacgcaatttatacctgtgccgatcaactactgacccggcagaacgaagtcctttacatgctggatttaacaaaggctaaagaactccatcaggaaataaaaaactactccaaaaaagagatagacatctttatcagaacagtaaccctgctggcctattcgcggataactcctgaagctgcctcgaatgagtttaagaaaaacaacctcattccgttactgctgcttctgccgactgatccccatcaacgcctgagcattttgcacctcttgaaaaaggtataaccatgatttactacgataatgcgtttcggttgcgtatccgtcacacaagtgtttaccagatccaccagcacctggattttttcatgcaggaacgtaagggagagaagctgccgtactcttttaaaatttttcccggtaccggggatgattcgttactcctggtccgcacagccacagctctggagttgccaggggagaaaaaaagagagcttattctctctgagggccatgaaatcaagttcattacgtcaatggccatctttcataaaggaacaaagtcagaaggccgtggccgacgccagtttgctccatccgaagaggctagttatcagttggccctcaccaaattagcgaaggctggttttaaacccggtcaaatcgtcgtcagtggcccgaaattcgtccatatcgtcaaaggaaatgctggacgcggttttacgctacccgtattcacggtacagggtaccgccataatcagcaatcaacaggaagctgaagttggaatcgtttatggcgtaggccctaaacgcgtatttggttgcggtttcatgcatctggcggggcagtagtcatgaatacatcagcggtatttgagtctgccggattgtcgttacgtaaggtccaacaggattatatcgaggctgcagctggtgcgctgactcaggatcataaagttgcactgattagtgctgaaacaggtgtaggaaaaacgctgggctatctggtaccggcgcttctgattctgctgaaaaacccagaggcaaaatttgtgatagccacgaattctcatgccctgatgcaccagatattcagaagcgatcgtcctctccttgaacagatagctgaacaatgcggcataaaagttactttttcccggcttatggggaaagcaaattacgtatccctggagaaagtacgtggactgttactcatggacgaatttaccgatctggatacggttaaggtccttgaaaaactcgctaactggtcaaaacctctggttgagtttgaagaagagtatggtgaactgccagcgcagatcacgccagagatggtcacctactccatctgggatgatatacaggacattgatgatattcgcctgaatgctctcagtgctaactttatagttacgacccatgcgatggtaatggtcgactgtatgtgtaatcaccgcatcctcggtgacaaagaaaatatgtacctcattattgatgaggcagacatttttgtagatatgcttgaggtctggaaacagcggcgcttcaacctcagagagttgaccagtgcgttcaatgaacatattccacgtaatggcgtgcatgtcatcgaccagttaatgaacgacgtgacttcgatagcgggcgatctgcatttttgtagtacgcctgcagcggttgccttgtttgacaatagctttaacgccttatcaaaggtagggcgggaaataaaaaatgaagcggcccggaaagctttctttgactgtatctacagctgggaaatgctcggattgtccggggggcaaaagggtgtaggcgtttccaataaacgtcgtgaaccagccctgatcgctgtaaacccgtttatcgggatgaatgtgggcagatactgcactcaatggcgtagtgcgttactgacgtcggctacgctctcaattaccagtaccccagagaccggaatggagtggttatgtaaagctctggggttaaccagcgatacgatttcaatcaggaaaatattctccccagacgtctatggctcaatgaagctgaccatcgccggtgctgattttccaaaggtgttcaatgacccgaaagaacagatattttcaggtcaatggttaaaggcagtagttgaacaattgtcctgtattcaggggccagctctggtattaactgccagccattatgaaaccaggatgattgccaatcagctgggtgaggtctcgcaaccagtttatattcagaaagcaggtcaggccctgtccgaaattattaaacagtatcaggagataccagggattcttatttctgccggtgcttctgttggtgtgagcccacgaggcgagaatggggaacagattttccaggatttaatcattacccggatacctttcttacctccggacagaatgaaggctgaaagcctttatgggtatctgaaggaacgaggctatagtcgtacctttgaggcagttaaccgtaacatctacctggataatttgcggaaagttattcgtaaagcaaagcagtctatagggcgggggattcgtagtgaaaatgataccgtcaggataattatcctcgatccgcgtttcccggaacctactgacctttcgtctaaacatcggtcgcttgaacacattattcccgttcgatttcgtcgtgcatatcgttcgtgtgaaattttatctccggcgtattgtgaagaggatatccagtgttaaattttaaaccgtatcgggtcatcatgtcttctctgacaccggtggtcatcagtgggatagccccatcgctggacggcattctgtatgaagcactgtctcaggcgatacccagtaacgagccaggagtcgtattggctcgtcttaaggaaatacttctattcaacgatgaactgggtgttttccatgcttcatctctacgttttggcataacgcccgaacaggggattggggcgacaacaagcgtacgttgcgattatctcagtcccgaaaaactgagcactgcaatgttctctcctcgtatccacaggggggtgtttacgcgtgtcctcctgaccgggggccccacgaagagaaggatgacaacccgtccagcttattctgcaccctatttaacgtttgattttgtcggctcttctgaggctgtagaaatactgcttaaccatgcccatgttggcgttggttatgactttttctctgcagctaatggagagtttaacaatgtgacaattcttcctctcgatatcgacacgagtatatccaacgagggtatggcattgcgtccggtacctgttaattcgggtctgaatggtatcaaaggagtatcaccacttattcctccctatttcgttggtgaaaagctaaacattgtccacccagcaccagttcgtactcaattgatttcttctttattgcgaggctaatttcatgagaactttaaacttcaacggtaaaatttcgactctggaaccactgactgtaacagtaaaaaatgcggtctcaacttccggccatcgcttgcctcgtaacggtggattcaatgcagccccgtactttccaggtaccagcattcggggaactcttcgtcatgctgcgcataaggtcattgtcgatcgtgtgggccttaatgcagacggaaaatcatccttcgacctggcagaacatttcatgctggcccagggggtggatatcaatggtgaagccgaaaccttcgcgccaggtgaaatcaatgctggtgctgaactacgtagcaaaaacccgttaatcagcttgtttggtcgttggggattaagcggcaaagttggtatagggaatgctatcccggatggtgataaccagtgggggatgtttggtggtggtgcccgctcaattatgtttcagcgtgacgaaagtctgatggagtttcttgagacagaccaggttgatcgtcttgaacgcctgctcgaggaacaggctgaggcaagtgtggatatctctcagatcaaaacagagcaagatgcactcaaaaaggcgatgaagtcggctgataaagacaccaaagctgagcttcaaatcaaagtacgggagctcgatgaaaaaattcaggcccgcaaagatcagaagcaggaatctcgcgagtcaattcgccgcccgattgacccgtatgaagcgtttatcaccggcgcagaactcagccatcgcatgagtattaaaaatgcgactgatgaggaagcagggcttttcatttctgcattaatccgctttgcagccgaaccacgttttggcggtcatgcgaatcataactgcggtctggtggaggctcactggacagttacgacctggaagccgggtgaactggtaccagttacacttggagaaatcgtcatcacaccgaatggtgttgagattaccggggacgagttgtttgctatggtaaaggcattcaatgaaaatcaatcttttgatttcactgcccgctaactccaaaagctggtggattttagtggcgctatttaatattttataatcaaccggttatttttagagtattccccccgtgtgcgggggttatcggtggggcgttgttgaataaatagatattatgctgcgggcctaccaaaacgtcggtctttcccaacgcaaaatcagtaggttaaggttaaagtcgggagctactcacaatagtgacaagcatctttgactaaagcaggcgcgccaaaacagcatgattccctattattcaacaaagcctatcggtggtgctctcaaccgtcacccgctggctggaagtattccccccgtgtgcgggggttatcggtcgtgttgtccacggttacccgctggctggaagtattccccccgcatgcgggggttatcggttaccaatggggaaaaatcttcatttgtaaatgtattccccccgcatgcgggggttatcggaacatcagtggaaatccactgcggcgtattctccccgcatgcgggggttatcggcgaaaacggcaaccttcataaaaacgtcttttgtattccccccgtgtgcgggggttatcggccgagattgagtaaagcaaagtaacggcggtggtattccccccgcatgcgggggttatcggcaggttatactggcaaaacgtcgatg

SEQ ID NO: 13 - skipped

SEQ ID NO: 14 - DNA, 85 bp, Escherichia coli
  source 1..85: mol_type = genomic DNA
aacctaaatatttgttgttaagctgcaatggaaacggtaaaagcggctagtatttaaagggatggatgacatctcagcgttgtcg

SEQ ID NO: 15 - DNA, 160 bp, synthetic construct
  source 1..160: mol_type = other DNA
cctgatgcgtgaacgtgacggacgtaaccaccgcgacatgtgtgtgctgttccgctgggcatgctgagctaacaccgtgcgtgttgacaattttacctctggcggtgataatggttgcagctagcaataattttgtttaactttaagaaggagatatacc

SEQ ID NO: 16 - DNA, 48 bp, synthetic construct
  source 1..48: mol_type = other DNA
agcggcagcgagactcccgggacctcagagtccgccacacccgaaagt

SEQ ID NO: 17 - protein, 16 aa, synthetic construct
SGSETPGTSESATPES

SEQ ID NO: 18 - DNA, 624 bp, Petromyzon marinus
  source 1..624: mol_type = other DNA
atgaccgacgctgagtacgtgagaatccatgagaagttggacatctacacgtttaagaaacagtttttcaacaacaaaaaatccgtgtcgcatagatgctacgttctctttgaattaaaacgacggggtgaacgtagagcgtgtttttggggctatgctgtgaataaaccacagagcgggacagaacgtggcattcacgccgaaatctttagcattagaaaagtcgaagaatacctgcgcgacaaccccggacaattcacgataaattggtactcatcctggagtccttgtgcagattgcgctgaaaagatcttagaatggtataaccaggagctgcgggggaacggccacactttgaaaatctgggcttgcaaactctattacgagaaaaatgcgaggaatcaaattgggctgtggaatctcagagataacggggttgggttgaatgtaatggtaagtgaacactaccaatgttgcaggaaaatattcatccaatcgtcgcacaatcaattgaatgagaatagatggcttgagaagactttgaagcgagctgaaaaacgacggagcgagttgtccattatgattcaggtaaaaatactccacaccactaagagtcctgctgtt

SEQ ID NO: 19 - protein, 208 aa, Petromyzon marinus
MTDAEYVRIHEKLDIYTFKKQFFNNKKSVSHRCYVLFELKRRGERRACFWGYAVNKPQSGTERGIHAEIFSIRKVEEYLRDNPGQFTINWYSSWSPCADCAEKILEWYNQELRGNGHTLKIWACKLYYEKNARNQIGLWNLRDNGVGLNVMVSEHYQCCRKIFIQSSHNQLNENRWLEKTLKRAEKRRSELSIMIQVKILHTTKSPAV

SEQ ID NO: 20 - DNA, 255 bp, Homo sapiens
  source 1..255: mol_type = other DNA
atgaccaacctttccgacatcatagagaaggaaacaggcaaacagttggtcatccaagagtcgatactcatgcttcctgaagaagttgaggaggtcattgggaataagccggaaagtgacattctcgtacacactgcgtatgatgagagcaccgatgagaacgtgatgctgctcacgtcagatgccccagagtacaaaccctgggctctggtgattcaggactctaatggagagaacaagatcaagatgctataa

SEQ ID NO: 21 - protein, 84 aa, Homo sapiens
MTNLSDIIEKETGKQLVIQESILMLPEEVEEVIGNKPESDILVHTAYDESTDENVMLLTSDAPEYKPWALVIQDSNGENKIKML

SEQ ID NO: 22 - DNA, 30 bp, synthetic construct
  source 1..30: mol_type = other DNA
tctggtggatctggaggttctggtggatct

SEQ ID NO: 23 - protein, 10 aa, synthetic construct
SGGSGGSGGS

SEQ ID NO: 24 - DNA, 213 bp, Escherichia coli
  source 1..213: mol_type = genomic DNA
gaccaaagccatgacaaaaacgcgtaacaaaagtgtctataatcacggcagaaaagtccacattgattatttgcacggcgtcacactttgctatgccatagcatttttatccataagattagcggatcctacctgacgctttttatcgcaactctctactgtttctccatacccgtttttttgggaattcgagctctaaggaggttataaaaa

SEQ ID NO: 25 - DNA, 32 bp, synthetic construct
  source 1..32: mol_type = other DNA
ggagacgtcatgtcaagctcataggcgtctcg

SEQ ID NO: 26 - DNA, 32 bp, synthetic construct
  source 1..32: mol_type = other DNA
acatacgcttcttgctgagtacgtgagttcac

SEQ ID NO: 27 - DNA, 32 bp, synthetic construct
  source 1..32: mol_type = other DNA
cagattgctggtcaggagcatattgatccgct

SEQ ID NO: 28 - DNA, 32 bp, synthetic construct
  source 1..32: mol_type = other DNA
aaggagatataccatggagcttttcactggcg

SEQ ID NO: 29 - DNA, 32 bp, synthetic construct
  source 1..32: mol_type = other DNA
ttcagcgtgtccggcgagggcgagggcgatgc

SEQ ID NO: 30 - DNA, 32 bp, synthetic construct
  source 1..32: mol_type = other DNA
ctgcccgtgccctggcccaccctcgtgaccac

SEQ ID NO: 31 - DNA, 32 bp, synthetic construct
  source 1..32: mol_type = other DNA
gagaagcgcgatcacatggtcctgctggagtt

SEQ ID NO: 32 - DNA, 32 bp, synthetic construct
  source 1..32: mol_type = other DNA
taccagatggcattgcgccatctggcagagtg

SEQ ID NO: 33 - DNA, 32 bp, synthetic construct
  source 1..32: mol_type = other DNA
aaagtcaggttgcgcaggcagggtaatcgggg

SEQ ID NO: 34 - DNA, 32 bp, synthetic construct
  source 1..32: mol_type = other DNA
tcacgtactcagcaagaagcgtatgtgtttgc

SEQ ID NO: 35 - DNA, 32 bp, synthetic construct
  source 1..32: mol_type = other DNA
acctctgtcagctcgctgacattccccgccag

SEQ ID NO: 36 - DNA, 32 bp, synthetic construct
  source 1..32: mol_type = other DNA
ttaaacaaaattattgctagctgcaaccatta

SEQ ID NO: 37 - DNA, 32 bp, synthetic construct
  source 1..32: mol_type = other DNA
ctccatggtatatctccttcttaaagttaaac

SEQ ID NO: 38 - DNA, 32 bp, synthetic construct
  source 1..32: mol_type = other DNA
cactgcacgccgtaggtcagggtggtcacgag

SEQ ID NO: 39 - DNA, 32 bp, synthetic construct
  source 1..32: mol_type = other DNA
tccagcaggaccatgtgatcgcgcttctcgtt

SEQ ID NO: 40 - DNA, 32 bp, synthetic construct
  source 1..32: mol_type = other DNA
cactctgccagatggcgcaatgccatctggta

SEQ ID NO: 41 - DNA, 32 bp, synthetic construct
  source 1..32: mol_type = other DNA
ctgactttgttgtcggcccggcgggcactcaa

SEQ ID NO: 42 - skipped

SEQ ID NO: 43 - DNA, 31 bp, synthetic construct
  source 1..31: mol_type = other DNA
ctcagtagatgttttcttgggtctaccgtta

SEQ ID NO: 44 - DNA, 618 bp, Tequatrovirus T4
  source 1..618: mol_type = other DNA
atgaaaagcggaatttatcagattaaaaatactttaaacaataaagtatatgtaggaagtgctaaagattttgaaaagagatggaagaggcattttaaagatttagaaaaaggatgccattcttctataaaacttcagaggtcttttaacaaacatggtaatgtgtttgaatgttctattttggaagaaattccatatgagaaagatttgattattgaacgagaaaatttttggattaaagagcttaattctaaaattaatggatacaatattgctgatgcaacgtttggtgatacatgttctacgcatccattaaaagaagaaattattaagaaacgttctgaaactgttaaagctaagatgcttaaacttggacctgatggtcggaaagctctttacagtaaacccggaagtaaaaacgggcgttggaatccagaaacccataagttttgtaagtgcggtgttcgcatacaaacttctgcttatacttgtagtaaatgcagaaatcgttcaggtgaaaataattcattctttaatcataagcattcagacataactaaatctaaaatatcagaaaagatgaaaggtaaaaagcctagtaatattaaaaagatttca

SEQ ID NO: 45 - protein, 206 aa, Tequatrovirus T4
MKSGIYQIKNTLNNKVYVGSAKDFEKRWKRHFKDLEKGCHSSIKLQRSFNKHGNVFECSILEEIPYEKDLIIERENFWIKELNSKINGYNIADATFGDTCSTHPLKEEIIKKRSETVKAKMLKLGPDGRKALYSKPGSKNGRWNPETHKFCKCGVRIQTSAYTCSKCRNRSGENNSFFNHKHSDITKSKISEKMKGKKPSNIKKIS

SEQ ID NO: 46 - DNA, 31 bp, synthetic construct; identical to SEQ ID NO: 43
  source 1..31: mol_type = other DNA

SEQ ID NO: 47 - DNA, 29 bp, synthetic construct
  source 1..29: mol_type = other DNA
ctcagtagatgttttcttgggtctaccgt

SEQ ID NO: 48 - DNA, 27 bp, synthetic construct
  source 1..27: mol_type = other DNA
ctcagtagatgttttcttgggtctacc

SEQ ID NO: 49 - DNA, 25 bp, synthetic construct
  source 1..25: mol_type = other DNA
ctcagtagatgttttcttgggtcta

SEQ ID NO: 50 - DNA, 23 bp, synthetic construct
  source 1..23: mol_type = other DNA
ctcagtagatgttttcttgggtc

SEQ ID NO: 51 - DNA, 21 bp, synthetic construct
  source 1..21: mol_type = other DNA
ctcagtagatgttttcttggg

SEQ ID NO: 52 - DNA, 19 bp, synthetic construct
  source 1..19: mol_type = other DNA
ctcagtagatgttttcttg

SEQ ID NO: 53 - DNA, 17 bp, synthetic construct
  source 1..17: mol_type = other DNA
ctcagtagatgttttct

SEQ ID NO: 54 - DNA, 15 bp, synthetic construct
  source 1..15: mol_type = other DNA
ctcagtagatgtttt

SEQ ID NO: 55 - DNA, 13 bp, synthetic construct
  source 1..13: mol_type = other DNA
ctcagtagatgtt

SEQ ID NO: 56 - DNA, 11 bp, synthetic construct
  source 1..11: mol_type = other DNA
ctcagtagatg

SEQ ID NO: 57-59 - skipped (3 entries)

SEQ ID NO: 60 - DNA, 33 bp, synthetic construct
  source 1..33: mol_type = other DNA
ctcagtagatgttttcttgggtctaccgttacg

SEQ ID NO: 61 - DNA, 35 bp, synthetic construct
  source 1..35: mol_type = other DNA
ctcagtagatgttttcttgggtctaccgttacgga

SEQ ID NO: 62 - DNA, 37 bp, synthetic construct
  source 1..37: mol_type = other DNA
ctcagtagatgttttcttgggtctaccgttacggatt

SEQ ID NO: 63 - DNA, 39 bp, synthetic construct
  source 1..39: mol_type = other DNA
ctcagtagatgttttcttgggtctaccgttacggattag

SEQ ID NO: 64 - DNA, 28 bp, synthetic construct
  source 1..28: mol_type = other DNA
ctcagtagatgttttcttgggtctaccg

SEQ ID NO: 65 - DNA, 30 bp, synthetic construct
  source 1..30: mol_type = other DNA
ctcagtagatgttttcttgggtctaccgtt

SEQ ID NO: 66 - DNA, 32 bp, synthetic construct
  source 1..32: mol_type = other DNA
ctcagtagatgttttcttgggtctaccgttac

SEQ ID NO: 67 - DNA, 34 bp, synthetic construct
  source 1..34: mol_type = other DNA
ctcagtagatgttttcttgggtctaccgttacgg

SEQ ID NO: 68 - DNA, 36 bp, synthetic construct
  source 1..36: mol_type = other DNA
ctcagtagatgttttcttgggtctaccgttacggat

SEQ ID NO: 69 - DNA, 32 bp, synthetic construct
  source 1..32: mol_type = other DNA
tcgtgttgtccacggttacccgctggctggaa

SEQ ID NO: 70 - DNA, 29 bp, synthetic construct
  source 1..29: mol_type = other DNA
gtattccccccgcatgcgggggttatcgg